European Patent Application EP 4 560 315 A2, published May 28, 2025. Title: Hybridizing all-LNA oligonucleotides. Applicant: F. Hoffmann-La Roche AG. Application EP. The sequence listing filed with the application follows.

SEQUENCE LISTING (70 sequences)

SEQ ID NO: 1-4 - skipped (4 entries)

SEQ ID NO: 5 - RNA, 10 nt, synthetic construct
  modified_base 2: mod_base = OTHER; note = thymine
  modified_base 6: mod_base = OTHER; note = thymine
  misc_feature 1..10: note = Single-stranded oligonucleotide consisting of either D-LNA or L-LNA monomers; in the sequence of nucleobases a signifies adenine, t signifies thymine, u signifies uracil, g signifies guanine, and any c is either cytosine or 5-methylcytosine.
  source 1..10: mol_type = other RNA
ctgcctgacg

SEQ ID NO: 6 - RNA, 10 nt, synthetic construct
  modified_base 3: mod_base = OTHER; note = thymine
  misc_feature 1..10: note = Single-stranded oligonucleotide consisting of either D-LNA or L-LNA monomers; in the sequence of nucleobases a signifies adenine, t signifies thymine, u signifies uracil, g signifies guanine, and any c is either cytosine or 5-methylcytosine.
  source 1..10: mol_type = other RNA
cgtcaggcag

SEQ ID NO: 7 - RNA, 12 nt, synthetic construct
  modified_base 4: mod_base = OTHER; note = thymine
  modified_base 8: mod_base = OTHER; note = thymine
  misc_feature 1..12: note = Single-stranded oligonucleotide consisting of either D-LNA or L-LNA monomers; in the sequence of nucleobases a signifies adenine, t signifies thymine, u signifies uracil, g signifies guanine, and any c is either cytosine or 5-methylcytosine.
  source 1..12: mol_type = other RNA
gactgcctgacg

SEQ ID NO: 8 - RNA, 12 nt, synthetic construct
  modified_base 3: mod_base = OTHER; note = thymine
  modified_base 11: mod_base = OTHER; note = thymine
  misc_feature 1..12: note = Single-stranded oligonucleotide consisting of either D-LNA or L-LNA monomers; in the sequence of nucleobases a signifies adenine, t signifies thymine, u signifies uracil, g signifies guanine, and any c is either cytosine or 5-methylcytosine.
  source 1..12: mol_type = other RNA
cgtcaggcagtc

SEQ ID NO: 9-16 - skipped (8 entries)

SEQ ID NO: 17 - RNA, 12 nt, synthetic construct
  misc_feature 1..12: note = Single-stranded oligonucleotide consisting of either D-LNA or L-LNA monomers; in the sequence of nucleobases a signifies adenine, t signifies thymine, u signifies uracil, g signifies guanine, and any c is either cytosine or 5-methylcytosine.
  source 1..12: mol_type = other RNA
caacacaccaac

SEQ ID NO: 18 - RNA, 10 nt, synthetic construct
  misc_feature 1..10: note = Single-stranded oligonucleotide consisting of either D-LNA or L-LNA monomers; in the sequence of nucleobases a signifies adenine, t signifies thymine, u signifies uracil, g signifies guanine, and any c is either cytosine or 5-methylcytosine.
  source 1..10: mol_type = other RNA
acacaccaac

SEQ ID NO: 19-22 - skipped (4 entries)

SEQ ID NO: 23 - RNA, 12 nt, synthetic construct
  modified_base 2..3: mod_base = OTHER; note = thymine
  modified_base 6: mod_base = OTHER; note = thymine
  modified_base 8: mod_base = OTHER; note = thymine
  modified_base 10..11: mod_base = OTHER; note = thymine
  misc_feature 1..12: note = Single-stranded oligonucleotide consisting of either D-LNA or L-LNA monomers; in the sequence of nucleobases a signifies adenine, t signifies thymine, u signifies uracil, g signifies guanine, and any c is either cytosine or 5-methylcytosine.
  source 1..12: mol_type = other RNA
gttggtgtgttg

SEQ ID NO: 24-30 - skipped (7 entries)

SEQ ID NO: 31 - RNA, 15 nt, synthetic construct
  modified_base 2..3: mod_base = OTHER; note = thymine
  modified_base 6: mod_base = OTHER; note = thymine
  modified_base 8: mod_base = OTHER; note = thymine
  modified_base 10..11: mod_base = OTHER; note = thymine
  modified_base 14: mod_base = OTHER; note = thymine
  misc_feature 1..15: note = Single-stranded oligonucleotide consisting of either D-LNA or L-LNA monomers; in the sequence of nucleobases a signifies adenine, t signifies thymine, u signifies uracil, g signifies guanine, and any c is either cytosine or 5-methylcytosine.
  source 1..15: mol_type = other RNA
gttggtgtgttggtg

SEQ ID NO: 32 - RNA, 15 nt, synthetic construct
  misc_feature 1..15: note = Single-stranded oligonucleotide consisting of either D-LNA or L-LNA monomers; in the sequence of nucleobases a signifies adenine, t signifies thymine, u signifies uracil, g signifies guanine, and any c is either cytosine or 5-methylcytosine.
  source 1..15: mol_type = other RNA
caccaacacaccaac

SEQ ID NO: 33-46 - skipped (14 entries)

SEQ ID NO: 47 - RNA, 15 nt, synthetic construct
  modified_base 3: mod_base = OTHER; note = thymine
  modified_base 11..12: mod_base = OTHER; note = thymine
  misc_feature 1..15: note = Single-stranded oligonucleotide consisting of either D-LNA or L-LNA monomers; in the sequence of nucleobases a signifies adenine, t signifies thymine, u signifies uracil, g signifies guanine, and any c is either cytosine or 5-methylcytosine.
  source 1..15: mol_type = other RNA
cgtcaggcagttcag

SEQ ID NO: 48 - RNA, 15 nt, synthetic construct
  modified_base 2: mod_base = OTHER; note = thymine
  modified_base 7: mod_base = OTHER; note = thymine
  modified_base 11: mod_base = OTHER; note = thymine
  misc_feature 1..15: note = Single-stranded oligonucleotide consisting of either D-LNA or L-LNA monomers; in the sequence of nucleobases a signifies adenine, t signifies thymine, u signifies uracil, g signifies guanine, and any c is either cytosine or 5-methylcytosine.
  source 1..15: mol_type = other RNA
ctgaactgcctgacg

SEQ ID NO: 49 - skipped

SEQ ID NO: 50 - RNA, 15 nt, synthetic construct
  modified_base 2..3: mod_base = OTHER; note = thymine
  modified_base 6: mod_base = OTHER; note = thymine
  modified_base 8: mod_base = OTHER; note = thymine
  modified_base 10..11: mod_base = OTHER; note = thymine
  modified_base 14: mod_base = OTHER; note = thymine
  misc_feature 1..15: note = Single-stranded oligonucleotide consisting of either D-LNA or L-LNA monomers; in the sequence of nucleobases a signifies adenine, t signifies thymine, u signifies uracil, g signifies guanine, and any c is either cytosine or 5-methylcytosine.
  source 1..15: mol_type = other RNA
gttggtgtgttggtg

SEQ ID NO: 51 - skipped

SEQ ID NO: 52 - RNA, 12 nt, synthetic construct
  misc_feature 1..12: note = Single-stranded oligonucleotide consisting of either D-LNA or L-LNA monomers; in the sequence of nucleobases a signifies adenine, t signifies thymine, u signifies uracil, g signifies guanine, and any c is either cytosine or 5-methylcytosine.
  source 1..12: mol_type = other RNA
caacacaccaac

SEQ ID NO: 53 - RNA, 12 nt, synthetic construct
  modified_base 2..3: mod_base = OTHER; note = thymine
  modified_base 6: mod_base = OTHER; note = thymine
  modified_base 8: mod_base = OTHER; note = thymine
  modified_base 10..11: mod_base = OTHER; note = thymine
  misc_feature 1..12: note = Single-stranded oligonucleotide consisting of either D-LNA or L-LNA monomers; in the sequence of nucleobases a signifies adenine, t signifies thymine, u signifies uracil, g signifies guanine, and any c is either cytosine or 5-methylcytosine.
  source 1..12: mol_type = other RNA
gttggtgtgttg

SEQ ID NO: 54 - RNA, 15 nt, synthetic construct
  misc_feature 1..15: note = Single-stranded oligonucleotide consisting of either D-LNA or L-LNA monomers; in the sequence of nucleobases a signifies adenine, t signifies thymine, u signifies uracil, g signifies guanine, and any c is either cytosine or 5-methylcytosine.
  source 1..15: mol_type = other RNA
caccaacacaccaac

SEQ ID NO: 55 - RNA, 15 nt, synthetic construct
  modified_base 3: mod_base = OTHER; note = thymine
  modified_base 11..12: mod_base = OTHER; note = thymine
  misc_feature 1..15: note = Single-stranded oligonucleotide consisting of either D-LNA or L-LNA monomers; in the sequence of nucleobases a signifies adenine, t signifies thymine, u signifies uracil, g signifies guanine, and any c is either cytosine or 5-methylcytosine.
  source 1..15: mol_type = other RNA
cgtcaggcagttcag

SEQ ID NO: 56-58 - skipped (3 entries)

SEQ ID NO: 59 - RNA, 20 nt, synthetic construct
  modified_base 4: mod_base = OTHER; note = thymine
  modified_base 14: mod_base = OTHER; note = thymine
  modified_base 20: mod_base = OTHER; note = thymine
  misc_feature 1..20: note = Single-stranded oligonucleotide consisting of either D-LNA or L-LNA monomers; in the sequence of nucleobases a signifies adenine, t signifies thymine, u signifies uracil, g signifies guanine, and any c is either cytosine or 5-methylcytosine.
  source 1..20: mol_type = other RNA
cagtggacgacgatagacat

SEQ ID NO: 60 - RNA, 20 nt, synthetic construct
  modified_base 2: mod_base = OTHER; note = thymine
  modified_base 4: mod_base = OTHER; note = thymine
  modified_base 6: mod_base = OTHER; note = thymine
  modified_base 8: mod_base = OTHER; note = thymine
  modified_base 11: mod_base = OTHER; note = thymine
  modified_base 14: mod_base = OTHER; note = thymine
  modified_base 19: mod_base = OTHER; note = thymine
  misc_feature 1..20: note = Single-stranded oligonucleotide consisting of either D-LNA or L-LNA monomers; in the sequence of nucleobases a signifies adenine, t signifies thymine, u signifies uracil, g signifies guanine, and any c is either cytosine or 5-methylcytosine.
  source 1..20: mol_type = other RNA
atgtctatcgtcgtccactg

SEQ ID NO: 61 - RNA, 20 nt, synthetic construct
  modified_base 7: mod_base = OTHER; note = thymine
  modified_base 15: mod_base = OTHER; note = thymine
  misc_feature 1..20: note = Single-stranded oligonucleotide consisting of either D-LNA or L-LNA monomers; in the sequence of nucleobases a signifies adenine, t signifies thymine, u signifies uracil, g signifies guanine, and any c is either cytosine or 5-methylcytosine.
  source 1..20: mol_type = other RNA
agaggatcgaggagtacagg

SEQ ID NO: 62 - RNA, 20 nt, synthetic construct
  modified_base 3: mod_base = OTHER; note = thymine
  modified_base 5: mod_base = OTHER; note = thymine
  modified_base 8: mod_base = OTHER; note = thymine
  modified_base 11: mod_base = OTHER; note = thymine
  modified_base 15: mod_base = OTHER; note = thymine
  modified_base 18: mod_base = OTHER; note = thymine
  modified_base 20: mod_base = OTHER; note = thymine
  misc_feature 1..20: note = Single-stranded oligonucleotide consisting of either D-LNA or L-LNA monomers; in the sequence of nucleobases a signifies adenine, t signifies thymine, u signifies uracil, g signifies guanine, and any c is either cytosine or 5-methylcytosine.
  source 1..20: mol_type = other RNA
cctgtactcctcgatcctct

SEQ ID NO: 63 - RNA, 20 nt, synthetic construct
  modified_base 6: mod_base = OTHER; note = thymine
  modified_base 15: mod_base = OTHER; note = thymine
  modified_base 18: mod_base = OTHER; note = thymine
  misc_feature 1..20: note = Single-stranded oligonucleotide consisting of either D-LNA or L-LNA monomers; in the sequence of nucleobases a signifies adenine, t signifies thymine, u signifies uracil, g signifies guanine, and any c is either cytosine or 5-methylcytosine.
  source 1..20: mol_type = other RNA
agaaatggacgagatgctaa

SEQ ID NO: 64 - RNA, 20 nt, synthetic construct
  modified_base 1..2: mod_base = OTHER; note = thymine
  modified_base 7: mod_base = OTHER; note = thymine
  modified_base 9: mod_base = OTHER; note = thymine
  modified_base 12: mod_base = OTHER; note = thymine
  modified_base 16..18: mod_base = OTHER; note = thymine
  modified_base 20: mod_base = OTHER; note = thymine
  misc_feature 1..20: note = Single-stranded oligonucleotide consisting of either D-LNA or L-LNA monomers; in the sequence of nucleobases a signifies adenine, t signifies thymine, u signifies uracil, g signifies guanine, and any c is either cytosine or 5-methylcytosine.
  source 1..20: mol_type = other RNA
ttagcatctcgtccatttct

SEQ ID NO: 65 - RNA, 20 nt, synthetic construct
  modified_base 3: mod_base = OTHER; note = thymine
  modified_base 8..9: mod_base = OTHER; note = thymine
  modified_base 11: mod_base = OTHER; note = thymine
  misc_feature 1..20: note = Single-stranded oligonucleotide consisting of either D-LNA or L-LNA monomers; in the sequence of nucleobases a signifies adenine, t signifies thymine, u signifies uracil, g signifies guanine, and any c is either cytosine or 5-methylcytosine.
  source 1..20: mol_type = other RNA
actgaacttgtgagaaacgc

SEQ ID NO: 66 - RNA, 20 nt, synthetic construct
  modified_base 4..6: mod_base = OTHER; note = thymine
  modified_base 8: mod_base = OTHER; note = thymine
  modified_base 15..16: mod_base = OTHER; note = thymine
  modified_base 20: mod_base = OTHER; note = thymine
  misc_feature 1..20: note = Single-stranded oligonucleotide consisting of either D-LNA or L-LNA monomers; in the sequence of nucleobases a signifies adenine, t signifies thymine, u signifies uracil, g signifies guanine, and any c is either cytosine or 5-methylcytosine.
  source 1..20: mol_type = other RNA
gcgtttctcacaagttcagt

SEQ ID NO: 67 - RNA, 20 nt, synthetic construct
  modified_base 2: mod_base = OTHER; note = thymine
  modified_base 9: mod_base = OTHER; note = thymine
  modified_base 18..20: mod_base = OTHER; note = thymine
  misc_feature 1..20: note = Single-stranded oligonucleotide consisting of either D-LNA or L-LNA monomers; in the sequence of nucleobases a signifies adenine, t signifies thymine, u signifies uracil, g signifies guanine, and any c is either cytosine or 5-methylcytosine.
  source 1..20: mol_type = other RNA
atggagagtcaggcaagttt

SEQ ID NO: 68 - RNA, 20 nt, synthetic construct
  modified_base 5..6: mod_base = OTHER; note = thymine
  modified_base 10: mod_base = OTHER; note = thymine
  modified_base 14: mod_base = OTHER; note = thymine
  modified_base 16: mod_base = OTHER; note = thymine
  modified_base 20: mod_base = OTHER; note = thymine
  misc_feature 1..20: note = Single-stranded oligonucleotide consisting of either D-LNA or L-LNA monomers; in the sequence of nucleobases a signifies adenine, t signifies thymine, u signifies uracil, g signifies guanine, and any c is either cytosine or 5-methylcytosine.
  source 1..20: mol_type = other RNA
aaacttgcctgactctccat

SEQ ID NO: 69 - RNA, 20 nt, synthetic construct
  modified_base 1: mod_base = OTHER; note = thymine
  modified_base 7: mod_base = OTHER; note = thymine
  modified_base 13: mod_base = OTHER; note = thymine
  modified_base 16: mod_base = OTHER; note = thymine
  misc_feature 1..20: note = Single-stranded oligonucleotide consisting of either D-LNA or L-LNA monomers; in the sequence of nucleobases a signifies adenine, t signifies thymine, u signifies uracil, g signifies guanine, and any c is either cytosine or 5-methylcytosine.
  source 1..20: mol_type = other RNA
tgaagatgcgagtgatgaac

SEQ ID NO: 70 - RNA, 20 nt, synthetic construct
  misc_feature 1..20: note = Single-stranded oligonucleotide consisting of either D-LNA or L-LNA monomers; in the sequence of nucleobases a signifies adenine, t signifies thymine, u signifies uracil, g signifies guanine, and any c is either cytosine or 5-methylcytosine.
  source 1..20: mol_type = other RNA
  modified_base 2..3: mod_base = OTHER; note = thymine
  modified_base 6: mod_base = OTHER; note = thymine
  modified_base 10: mod_base = OTHER; note = thymine
  modified_base 15: mod_base = OTHER; note = thymine
  modified_base 17..18: mod_base = OTHER; note = thymine
gttcatcactcgcatcttca